European Patent Specification EP 3 559 230 B1, published September 6, 2023. Title: METHODS FOR INCREASING THE EFFICIENCY OF HOMOLOGY DIRECTED REPAIR (HDR) IN THE CELLULAR GENOME. Applicant: Bristol-Myers Squibb Company. The sequence listing filed with the application follows.

SEQUENCE LISTING (18 sequences)

SEQ ID NO: 1 - DNA, 20 bp, Artificial Sequence
  oligonucleotide
tgggtttccaggaagaattg

SEQ ID NO: 2 - DNA, 20 bp, Artificial Sequence
  oligonucleotide
tccctctcaaaagcaaaagg

SEQ ID NO: 3 - DNA, 23 bp, Artificial Sequence
  oligonucleotide
ggtttaccattgcttgttcagag

SEQ ID NO: 4 - DNA, 22 bp, Artificial Sequence
  oligonucleotide
tgccctaaactaaaccaacaaa

SEQ ID NO: 5 - DNA, 22 bp, Artificial Sequence
  oligonucleotide
tgccctaaactaaaccaacaaa

SEQ ID NO: 6 - DNA, 22 bp, Artificial Sequence
  oligonucleotide
cagaccaagaagcattcaggaa

SEQ ID NO: 7 - DNA, 19 bp, Artificial Sequence
  oligonucleotide
atgctgccaaaattatcaa

SEQ ID NO: 8 - DNA, 18 bp, Artificial Sequence
  oligonucleotide
aaaagctctccgcaagag

SEQ ID NO: 9 - DNA, 20 bp, Artificial Sequence
  oligonucleotide
acaccaaaaagctttctgct

SEQ ID NO: 10 - DNA, 20 bp, Artificial Sequence
  oligonucleotide
aaaagctttctgctaggggt

SEQ ID NO: 11 - DNA, 20 bp, Artificial Sequence
  oligonucleotide
gtttggagaggaaagtggcg

SEQ ID NO: 12 - DNA, 20 bp, Artificial Sequence
  oligonucleotide
agaacgttcgtggttccgtg

SEQ ID NO: 13 - DNA, 177 bp, Artificial Sequence
  oligonucleotide
ttggtttccaggggggcattctcagtggtgagaagatgtatgaaaattcctactggacaagaatatgctgccaggattatcaacaccaaaaagctctccgcaagaggtgggtattttcaaccacatatattggttaattttgtatttgtcatgttgattataggttctgttgtatgt

SEQ ID NO: 14 - DNA, 161 bp, Artificial Sequence
  oligonucleotide
ttataactacatgatatatttacatacaacagaacctataatcaacatgacaaatacaaaattaaccaatatatgtggttgaaaatacccacctcttgcggagagctttttggtgttgataatcctggcagcatattcttgtccagtaggaattttcatac

SEQ ID NO: 15 - DNA, 175 bp, Artificial Sequence
  oligonucleotide
ctttaggtttaccattgcttgttcagagaacaattgcgagaactattgtgttacaagaaagcattggcaaaggccgatttggagaagtttggaggggcaaatggcggggagaagaagttgctgttaagatattctcctctagagaagaacgttcgtggttccgtgaggcagagat

SEQ ID NO: 16 - DNA, 157 bp, Artificial Sequence
  oligonucleotide
taacattacagtttgataaatctctgcctcacggaaccacgaacgttcttctctagaggagaatatcttaacagcaacttcttctccccgccatttgcccctccaaacttctccaaatcggcctttgccaatgctttcttgtaacacaatagttctc

SEQ ID NO: 17 - DNA, 179 bp, Artificial Sequence
  oligonucleotide
gcattggcaaaggtcgatttggagaagtttggagaggaaagtggcggggagaagaagttgctgttaagatattttcctctagagaagaacgttcgtggtttcgagaagcagagatttatcaaactgtaatgttacgtcatgaaaacatcctgggatttatagcagcagacaataaaggt

SEQ ID NO: 18 - DNA, 156 bp, Artificial Sequence
  oligonucleotide
agcaaatgttacagacctttattgtctgctgctataaatcccaggatgttttcatgacgtaacattacagtttgataaatctctgcttctcgaaaccacgaacgttcttctctagaggaaaatatcttaacagcaacttcttctccccgccacttt